European Patent Specification EP 3 498 847 B1, published September 23, 2026. Title: Vaccine composition comprising recombinant protein for preventing swine mycoplasma infection. Applicant: Innovac. The sequence listing filed with the application follows.

SEQUENCE LISTING (14 sequences)

SEQ ID NO: 1 - protein, 274 aa, artificial sequence
  Mycoplasma hyopneumoniae rP97 protein sequence
MGIPTKEGKREEVDKKVKELDNKIKGILPQPPAAKPEAAKPVAAKPEAAKPVAAKPEAAKPEAAKPVAAKPEAAKPVAAKPEAAKPVATNTNTGFSLTNKPKEDYFPMAFSYKLEYTDENKLSLKTPEINVFLELVHQSEYEEQKIIKELDKTVLNLQYQFQEVKVTSEQYQKLSHPMMTEGSPNQGKKGEGTPNQGKKAEGAPNQGKKAEGAPSQGKKAEGASNQQSPTTKGGRADPAFLYKVVINSKLEGKPIPNPLLGLDSTRTGHHHHHH

SEQ ID NO: 2 - DNA, 825 bp, artificial sequence
  Mycoplasma hyopneumoniae rP97 DNA sequence
atggggatccctacaaaagaaggtaaaagagaagaagtagataaaaaagttaaagaattagataataaaataaaaggtatattacctcagcccccagcagctaaaccagaagcagcaaaaccagtagcagctaaacctgaagcagcaaaaccagtagcggctaaacctgaagcagcaaaacctgaagcagcaaaaccagtagcggctaaacctgaagcagcaaaaccagtagcagctaaacctgaagcagcaaaaccagttgctactaatactaatactggcttttcacttacaaataaaccaaaagaagactatttcccaatggcttttagttataaattagaatatactgacgaaaataaattaagcctaaaaacaccggaaattaatgtatttttagaactagttcatcaaagcgagtatgaagaacaaaaaataataaaggaactagataaaactgttttaaatcttcaatatcaattccaggaagtcaaggtaactagtgaacaatatcagaaacttagccacccaatgatgaccgagggatctcctaatcaaggtaaaaaaggagaaggaactcctaaccaaggcaaaaaagccgaaggcgctcctaaccaaggcaaaaaagccgaaggcgcacctagtcaagggaaaaaagcagagggtgcttctaatcaacaaagcccaactaccaagggtgggcgcgccgacccagctttcttgtacaaagtggtgatcaattcgaagcttgaaggtaagcctatccctaaccctctcctcggtctcgattctacgcgtaccggtcatcatcaccatcaccattga

SEQ ID NO: 3 - DNA, 25 bp, artificial sequence
  LTB Forward primer
caccatggctccccagactattaca

SEQ ID NO: 4 - DNA, 21 bp, artificial sequence
  LTB Reverse primer
ctggatccccatactgattgc

SEQ ID NO: 5 - DNA, 26 bp, artificial sequence
  R1 Forward primer
caccatggggatccctacaaaagaag

SEQ ID NO: 6 - DNA, 22 bp, artificial sequence
  R1  Reverse primer
gccaagcttagtagcaactggt

SEQ ID NO: 7 - DNA, 26 bp, artificial sequence
  R1 Forward primer
caccatggggatccctacaaaagaag

SEQ ID NO: 8 - DNA, 18 bp, artificial sequence
  2Rs Reverse primer
ggtagttgggctttgttg

SEQ ID NO: 9 - DNA, 25 bp, artificial sequence
  LTB Forward primer
caccatggctccccagactattaca

SEQ ID NO: 10 - DNA, 22 bp, artificial sequence
  R1 Reverse primer
gccaagcttagtagcaactggt

SEQ ID NO: 11 - DNA, 25 bp, artificial sequence
  LTB Forward primer
caccatggctccccagactattaca

SEQ ID NO: 12 - DNA, 18 bp, artificial sequence
  2RsR
ggtagttgggctttgttg

SEQ ID NO: 13 - protein, 380 aa, artificial sequence
  Mycoplasma hyopneumoniae rP97m protein sequence
MHHHHHHSSGLVPRGSGMKETAAAKFERQHMDSPDLGTDDDDKAMADIGSEFAPQTITELCSEYRNTQIYTINDKILSYTESMAGKREMVIITFKSGATFQVEVPGSQHIDSQKKAIERMKDTLRIAYLTETKIDKLCVWNNKTPNSIAAISLEGIPTKEGKREEVDKKVKELDNKIKGILPQPPAAKPEAAKPVAAKPEAAKPVAAKPEAAKPEAAKPVAAKPEAAKPVAAKPEAAKPVATNEGTPNQGKKAEGAPNQGKKAEGAPSQGKKAEGASNQQSPTTELTNYLPELGKKIDEIIKKQGKNWKTEVELIEDNIAGDAKLLYFVLRDDSKSGDPKKSSLKVKITVKQSNNNQELKSKQACGRTRAPPPPPLRSGC

SEQ ID NO: 14 - DNA, 1143 bp, artificial sequence
  Mycoplasma hyopneumoniae rP97m DNA sequence
atgcaccatcatcatcatcattcttctggtctggtgccacgcggttctggtatgaaagaaaccgctgctgctaaattcgaacgccagcacatggacagcccagatctgggtaccgacgacgacgacaaggccatggctgatatcggatccgaattcgctccccagactattacagaactatgttcggaatatcgcaacacacaaatatatacgataaatgacaaaatactatcatatacggaatcgatggcaggcaaaagagaaatggttatcattacatttaagagcggcgcaacatttcaggtcgaagtcccgggcagtcaacatatagactcccaaaaaaaagccattgaaaggatgaaggacacattaagaatcgcatatctgaccgagaccaaaattgataaattatgtgtatggaataataaaacccccaattcaattgcggcaatcagtctcgaggggatccctacaaaagaaggtaaaagagaagaagtagataaaaaagttaaagaattagataataaaataaaaggtatattacctcagcccccagcagctaaaccagaagcagcaaaaccagtagcagctaaacctgaagcagcaaaaccagtagcggctaaacctgaagcagcaaaacctgaagcagcaaaaccagtagcggctaaacctgaagcagcaaaaccagtagcagctaaacctgaagcagcaaaaccagttgctactaatgaaggaactcctaaccaaggcaaaaaagccgaaggcgctcctaaccaaggcaaaaaagccgaaggcgcacctagtcaagggaaaaaagcagagggtgcttctaatcaacaaagcccaactaccgaattaactaattaccttcctgaattaggtaaaaaaattgacgaaatcattaaaaaacaaggtaaaaattggaaaacagaggttgaactaatcgaggataatatcgctggagatgctaaattgctatactttgtcctaagggatgattcaaaatccggtgatcctaaaaaatcaagtctaaaagttaaaataacagtaaaacaaagtaataataatcaggaattaaaatctaaacaagcttgcggccgcactcgagcaccaccaccaccaccactgagatccggctgctaa